European Patent Application EP 4 190 910 A1, published June 7, 2023. Title: Method for loading nucleic acid molecule on solid support. Applicant: MGI TECH CO., LTD. The sequence listing filed with the application follows.

SEQUENCE LISTING (4 sequences)

SEQ ID NO: 1 - DNA, 58 bp, artificial
  Nucleic acid strand of the library linker
agtcggaggccaagcggtcttaggaagacaatccttttgtacaactccttggctcaca

SEQ ID NO: 2 - DNA, 38 bp, artificial
  Nucleic acid strand of the library linker
ttgtcttcctaaggaacgacatggctacgatccgactt

SEQ ID NO: 3 - DNA, 24 bp, artificial
  RCA primer
gccatgtcgttctgtgagccaagg

SEQ ID NO: 4 - DNA, 32 bp, artificial
  Sequencing primer
gctcacagaacgacatggctacgatccgactt